European Patent Application EP 4 124 659 A1, published February 1, 2023. Title: APTAMERS AGAINST THE HEPATITIS C VIRUS CORE PROTEIN. Applicant: Consejo Superior de Investigaciones Científicas (CSIC) Instituto Nacional de Técnica Aeroespacial (INTA) FUNDACIÓN PARA LA INVESTIGACIÓN BIOMÉDICA DEL HOSPITAL UNIVERSITARIO RAMÓN Y CAJAL (IRYCIS) Aptus Biotech S.L. The sequence listing filed with the application follows.

SEQUENCE LISTING (51 sequences)

SEQ ID NO: 1 - DNA, 74 bp, Artificial Sequence
  consensus sequence with 74 nucleotides
gcggatsmagactggtgtdbnnnnnnbnbnnnnhbnnnndnbhnnhnbhnhybndbgccctaaakacragcwwc

SEQ ID NO: 2 - DNA, 75 bp, Artificial Sequence
  consensus sequence with 75 nucleotides
gcggatsmagactggtgtdbnnnnnnbnbnnnnhbnnnndnbhnnhnbhnhybndbbgccctaaakacragcwwc

SEQ ID NO: 3 - DNA, 76 bp, Artificial Sequence
  consensus sequence with 76 nucleotides
gcggatsmagactggtgtdbnnnnnnbnbnnnnhbnnnndnbhnnhnbhnhybndbbbgccctaaakacragcwwc

SEQ ID NO: 4 - DNA, 77 bp, Artificial Sequence
  consensus sequence with 77 nucleotides
gcggatsmagactggtgtdbnnnnnnbnbnnnnhbnnnndnbhnnhnbhnhybndbbbgccctaaakagcragcwwc

SEQ ID NO: 5 - DNA, 74 bp, Artificial Sequence
  consensus sequence of the aptamers Apt-HCVcore_01 to Apt-HCVcore_08 with 74 nucleotides
gcggatccagactggtgtrbnnnnnnbnbnnnbhbnnnndnbhnnhnbhnhybnwbgccctaaagacaagcttc

SEQ ID NO: 6 - DNA, 75 bp, Artificial Sequence
  consensus sequence of the aptamers Apt-HCVcore_01 to Apt-HCVcore_08 with 75 nucleotides
gcggatccagactggtgtrbnnnnnnbnbnnnbhbnnnndnbhnnhnbhnhybnwbbgccctaaagacaagcttc

SEQ ID NO: 7 - DNA, 76 bp, Artificial Sequence
  consensus sequence of the aptamers Apt-HCVcore_01 to Apt-HCVcore_08 with 76 nucleotides
gcggatccagactggtgtrbnnnnnnbnbnnnbhbnnnndnbhnnhnbhnhybnwbbbgccctaaagacaagcttc

SEQ ID NO: 8 - DNA, 76 bp, Artificial Sequence
  consensus sequence of the aptamers Apt-HCVcore_09 to Apt-HCVcore_11 with 76 nucleotides
gcggatgaagactggtgtkbmryhhyybysbcwykhwmytmthykwhchhtccvkysbgccctaaatacgagcaac

SEQ ID NO: 9 - DNA, 77 bp, Artificial Sequence
  consensus sequence of the aptamers Apt-HCVcore_09 to Apt-HCVcore_11 with 77 nucleotides
gcggatgaagactggtgtkbmryhhyybysbcwykhwmytmthykwhchhtccvkysbgccctaaatagcgagcaac

SEQ ID NO: 10 - DNA, 76 bp, Artificial Sequence
  Apt-HCVcore_01
gcggatccagactggtgtgccgtatccctcccttgtaattatttgttccatccgttccgccctaaagacaagcttc

SEQ ID NO: 11 - DNA, 76 bp, Artificial Sequence
  Apt-HCVcore_02
gcggatccagactggtgtgtgcgggtgggtgggtggtttgttctgctgtgttgttgtggccctaaagacaagcttc

SEQ ID NO: 12 - DNA, 74 bp, Artificial Sequence
  Apt-HCVcore_03
gcggatccagactggtgtatcttttgcatgacgactatttactaacttttctctaggccctaaagacaagcttc

SEQ ID NO: 13 - DNA, 75 bp, Artificial Sequence
  Apt-HCVcore_04
gcggatccagactggtgtagttcgggcttatatatacgaacccttagtaatccatgggccctaaagacaagcttc

SEQ ID NO: 14 - DNA, 76 bp, Artificial Sequence
  Apt-HCVcore_05
gcggatccagactggtgtggggtttctgtgtaccctggctgcagacgtatattttcgggccctaaagacaagcttc

SEQ ID NO: 15 - DNA, 76 bp, Artificial Sequence
  Apt-HCVcore_06
gcggatccagactggtgtggtggtaattttgtgtctggtttgttctctttctcgttgtgccctaaagacaagcttc

SEQ ID NO: 16 - DNA, 75 bp, Artificial Sequence
  Apt-HCVcore_07
gcggatccagactggtgtgtggaatgtgtggtgttcacggtgtaattctttttttcggccctaaagacaagcttc

SEQ ID NO: 17 - DNA, 76 bp, Artificial Sequence
  Apt-HCVcore_08
gcggatccagactggtgtgtaacccttgccgctctctactctacgtacactccctcgggccctaaagacaagcttc

SEQ ID NO: 18 - DNA, 76 bp, Artificial Sequence
  Apt-HCVcore_09
gcggatgaagactggtgtgccgtatccctcccttgtaattatttgttccatccgttccgccctaaatacgagcaac

SEQ ID NO: 19 - DNA, 77 bp, Artificial Sequence
  Apt-HCVcore_10
gcggatgaagactggtgtgtaacccttgccgctctctactctacgtacactccctcgggccctaaatagcgagcaac

SEQ ID NO: 20 - DNA, 76 bp, Artificial Sequence
  Apt-HCVcore_11
gcggatgaagactggtgttgcactaccttgtcatgaacttctcctacctttccagcctgccctaaatacgagcaac

SEQ ID NO: 21 - DNA, 74 bp, Artificial Sequence
  consensus complementary reverse sequence of SEQ ID NO: 1
gwwgctygtmtttagggcvhnvrdndvndnndvnhnnnnvdnnnnvnvnnnnnnvhacaccagtctksatccgc

SEQ ID NO: 22 - DNA, 75 bp, Artificial Sequence
  consensus complementary reverse sequence of SEQ ID NO: 2
gwwgctygtmtttagggcvvhnvrdndvndnndvnhnnnnvdnnnnvnvnnnnnnvhacaccagtctksatccgc

SEQ ID NO: 23 - DNA, 76 bp, Artificial Sequence
  consensus complementary reverse sequence of SEQ ID NO: 3
gwwgctygtmtttagggcvvvhnvrdndvndnndvnhnnnnvdnnnnvnvnnnnnnvhacaccagtctksatccgc

SEQ ID NO: 24 - DNA, 77 bp, Artificial Sequence
  consensus complementary reverse sequence of SEQ ID NO: 4
gwwgctygctmtttagggcvvvhnvrdndvndnndvnhnnnnvdnnnnvnvnnnnnnvhacaccagtctksatccgc

SEQ ID NO: 25 - DNA, 74 bp, Artificial Sequence
  consensus complementary reverse sequence of SEQ ID NO: 5
gaagcttgtctttagggcvwnvrdndvndnndvnhnnnnvdvnnnvnvnnnnnnvyacaccagtctggatccgc

SEQ ID NO: 26 - DNA, 75 bp, Artificial Sequence
  consensus complementary reverse sequence of SEQ ID NO: 6
gaagcttgtctttagggcvvwnvrdndvndnndvnhnnnnvdvnnnvnvnnnnnnvyacaccagtctggatccgc

SEQ ID NO: 27 - DNA, 76 bp, Artificial Sequence
  consensus complementary reverse sequence of SEQ ID NO: 7
gaagcttgtctttagggcvvvwnvrdndvndnndvnhnnnnvdvnnnvnvnnnnnnvyacaccagtctggatccgc

SEQ ID NO: 28 - DNA, 76 bp, Artificial Sequence
  consensus complementary reverse sequence of SEQ ID NO: 8
gttgctcgtatttagggcvsrmbggaddgdwmrdakarkwdmrwgvsrvrrddrykvmacaccagtcttcatccgc

SEQ ID NO: 29 - DNA, 77 bp, Artificial Sequence
  consensus complementary reverse sequence of SEQ ID NO: 9
gttgctcgctatttagggcvsrmbggaddgdwmrdakarkwdmrwgvsrvrrddrykvmacaccagtcttcatccgc

SEQ ID NO: 30 - DNA, 76 bp, Artificial Sequence
  Apt-HCVcore_01_reverse complementary
gaagcttgtctttagggcggaacggatggaacaaataattacaagggagggatacggcacaccagtctggatccgc

SEQ ID NO: 31 - DNA, 76 bp, Artificial Sequence
  Apt-HCVcore_02_reverse complementary
gaagcttgtctttagggccacaacaacacagcagaacaaaccacccacccacccgcacacaccagtctggatccgc

SEQ ID NO: 32 - DNA, 74 bp, Artificial Sequence
  Apt-HCVcore_03_reverse complementary
gaagcttgtctttagggcctagagaaaagttagtaaatagtcgtcatgcaaaagatacaccagtctggatccgc

SEQ ID NO: 33 - DNA, 75 bp, Artificial Sequence
  Apt-HCVcore_04_reverse complementary
gaagcttgtctttagggcccatggattactaagggttcgtatatataagcccgaactacaccagtctggatccgc

SEQ ID NO: 34 - DNA, 76 bp, Artificial Sequence
  Apt-HCVcore_05_reverse complementary
gaagcttgtctttagggcccgaaaatatacgtctgcagccagggtacacagaaaccccacaccagtctggatccgc

SEQ ID NO: 35 - DNA, 76 bp, Artificial Sequence
  Apt-HCVcore_06_reverse complementary
gaagcttgtctttagggcacaacgagaaagagaacaaaccagacacaaaattaccaccacaccagtctggatccgc

SEQ ID NO: 36 - DNA, 75 bp, Artificial Sequence
  Apt-HCVcore_07_reverse complementary
gaagcttgtctttagggccgaaaaaaagaattacaccgtgaacaccacacattccacacaccagtctggatccgc

SEQ ID NO: 37 - DNA, 76 bp, Artificial Sequence
  Apt-HCVcore_08_reverse complementary
gaagcttgtctttagggcccgagggagtgtacgtagagtagagagcggcaagggttacacaccagtctggatccgc

SEQ ID NO: 38 - DNA, 76 bp, Artificial Sequence
  Apt-HCVcore_09_reverse complementary
gttgctcgtatttagggcggaacggatggaacaaataattacaagggagggatacggcacaccagtcttcatccgc

SEQ ID NO: 39 - DNA, 77 bp, Artificial Sequence
  Apt-HCVcore_10_reverse complementary
gttgctcgctatttagggcccgagggagtgtacgtagagtagagagcggcaagggttacacaccagtcttcatccgc

SEQ ID NO: 40 - DNA, 76 bp, Artificial Sequence
  Apt-HCVcore_11_reverse complementary
gttgctcgtatttagggcaggctggaaaggtaggagaagttcatgacaaggtagtgcaacaccagtcttcatccgc

SEQ ID NO: 41 - protein, 122 aa, Artificial Sequence
  amino acids 1 to 122 of the HCV core protein (genotype 1)
MSTNPKPQRKTKRNTNRRPQDVKFPGGGQIVGGVYLLPRRGPRLGVRATRKTSERSQPRGRRQPIPKARRPEGRTWAQPGYPWPLYGNEGCGWAGWLLSPRGSRPSWGPTDPRRRSRNLGKV

SEQ ID NO: 42 - protein, 191 aa, Artificial Sequence
  HCV core protein (genotype 1)
MSTNPKPQRKTKRNTNRRPQDVKFPGGGQIVGGVYLLPRRGPRLGVRATRKTSERSQPRGRRQPIPKARRPEGRTWAQPGYPWPLYGNEGCGWAGWLLSPRGSRPSWGPTDPRRRSRNLGKVIDTLTCGFADLMGYIPLVGAPLGGAARALAHGVRVLEDGVNYATGNLPGCSFSIFLLALLSCLTVPASA

SEQ ID NO: 43 - protein, 191 aa, Artificial Sequence
  HCV core protein (genotype 2)
MSTNPKPQRLTKRNTNRRPQNVKFPGGGQIVGGVYLLPRRGPRVGVRATRKTSERSQPRGRRQPIPKDRRSTGKSWGKPGYPWPLYGNEGLGWAGWLLSPRGSRPTWGPNDPRHRSRNVGKVIDTITCGFADLMGYIPVVGAPVGGVARALAHGVRVLEDGINYATRNLPGCSFSIFLLALLSCISIPVSA

SEQ ID NO: 44 - protein, 189 aa, Artificial Sequence
  HCV core protein (genotype 3)
MSTLPKPQRQTKRNTRRPQNVKFPGGGQIVGGVYVLPRRGPRLGVRAVRKTSERSQPRGRRKPTPKARPGGRSWAQPGYPWPLYGNEGCGWAGWLLSPRGSRPNWGPNDPRRRSRNLGKVIDTLTCGFADLMGYIPLIGAPVGGVARALAHGVRALEDGINFATGNLPGCSFSIFLLALFSCLIHPAAS

SEQ ID NO: 45 - protein, 191 aa, Artificial Sequence
  HCV core protein (genotype 4)
MSTNPKPQRKTKRNTNRRPMDVKFPGGGQIVGGVYLLPRRGPRLGVRATRKTSERSQPRGRRQPIPKARRSEGRSWAQPGYPWPLYGNEGCGWAGWLLSPRGSRPSWGPNDPRRRSRNLGKVIDTLTCGFADLMGYIPLVGAPVGGVARALAHGVRAVEDGINYATGNLPGCSFSIFLLALLSCLTVPTSA

SEQ ID NO: 46 - DNA, 18 bp, Artificial Sequence
  5´-end SEQ ID NO: 5
gcggatccagactggtgt

SEQ ID NO: 47 - DNA, 18 bp, Artificial Sequence
  3´-end SEQ ID NO: 5
gccctaaagacaagcttc

SEQ ID NO: 48 - DNA, 18 bp, Artificial Sequence
  5´-end SEQ ID NO: 8
gcggatgaagactggtgt

SEQ ID NO: 49 - DNA, 18 bp, Artificial Sequence
  3´-end SEQ ID NO: 8
gccctaaatacgagcaac

SEQ ID NO: 50 - DNA, 76 bp, Artificial Sequence
  D-ACTG
gcggatccagactggtgtactgactgactgactgactgactgactgactgactgactggccctaaagacaagcttc

SEQ ID NO: 51 - RNA, 76 nt, Artificial Sequence
  R-ACUG
gcggauccagacugguguacugacugacugacugacugacugacugacugacugacuggcccuaaagacaagcuuc